European Patent Application EP 4 169 946 A1, published April 26, 2023. Title: ANTIBODIES BINDING SPECIFICALLY TO NT-PROBNP AND USE THEREOF. Applicant: BIONOTE, INC. The sequence listing filed with the application follows.

SEQUENCE LISTING (9 sequences)

SEQ ID NO: 1 - protein, 85 aa, synthetic construct
HPLGGRSPASEASEASEASGLWAVQELLGRLKDAVSELQAEQLALEPLHRSHSPAEAPEAGGTPRGVLAPHDSVLQALRRLRSPK

SEQ ID NO: 2 - skipped

SEQ ID NO: 3 - protein, 7 aa, synthetic construct
HPLGGRS

SEQ ID NO: 4 - protein, 9 aa, synthetic construct
GFSLSTSGV

SEQ ID NO: 5 - protein, 5 aa, synthetic construct
WWDDD

SEQ ID NO: 6 - protein, 10 aa, synthetic construct
MDDYNYAFDY

SEQ ID NO: 7 - protein, 16 aa, synthetic construct
KSSQSLLYSNGKTYLN

SEQ ID NO: 8 - protein, 7 aa, synthetic construct
LVSKLDS

SEQ ID NO: 9 - protein, 9 aa, synthetic construct
VQGTHFPLT